European Patent Specification EP 3 850 363 B1, published January 22, 2025. Title: Methods for high throughput peptide-MHC affinity screening for TCR ligands. Applicant: Immatics Biotechnologies GmbH. The sequence listing filed with the application follows.

SEQUENCE LISTING (325 sequences)

SEQ ID NO: 1 - protein, 9 aa, Homo sapiens
ALYNVLAKV

SEQ ID NO: 2 - protein, 6 aa, Homo sapiens
APPVAG

SEQ ID NO: 3 - protein, 9 aa, Homo sapiens
SLLMWITQC

SEQ ID NO: 4 - protein, 9 aa, Homo sapiens
SLLMWITQV

SEQ ID NO: 5 - protein, 9 aa, Homo sapiens
SLYNTVATL

SEQ ID NO: 6 - protein, 365 aa, Homo sapiens
MAVMAPRTLLLLLSGALALTQTWAGSHSMRYFFTSVSRPGRGEPRFIAVGYVDDTQFVRFDSDAASQKMEPRAPWIEQEGPEYWDQETRNMKAHSQTDRANLGTLRGYYNQSEDGSHTIQIMYGCDVGPDGRFLRGYRQDAYDGKDYIALNEDLRSWTAADMAAQITKRKWEAVHAAEQRRVYLEGRCVDGLRRYLENGKETLQRTDPPKTHMTHHPISDHEATLRCWALGFYPAEITLTWQRDGEDQTQDTELVETRPAGDGTFQKWAAVVVPSGEEQRYTCHVQHEGLPKPLTLRWELSSQPTIPIVGIIAGLVLLGAVITGAVVAAVMWRRKSSDRKGGSYTQAASSDSAQGSDVSLTACKV

SEQ ID NO: 7 - protein, 362 aa, Homo sapiens
MLVMAPRTVLLLLSAALALTETWAGSHSMRYFYTSVSRPGRGEPRFISVGYVDDTQFVRFDSDAASPREEPRAPWIEQEGPEYWDRNTQIYKAQAQTDRESLRNLRGYYNQSEAGSHTLQSMYGCDVGPDGRLLRGHDQYAYDGKDYIALNEDLRSWTAADTAAQITQRKWEAAREAEQRRAYLEGECVEWLRRYLENGKDKLERADPPKTHVTHHPISDHEATLRCWALGFYPAEITLTWQRDGEDQTQDTELVETRPAGDRTFQKWAAVVVPSGEEQRYTCHVQHEGLPKPLTLRWEPSSQSTVPIVGIVAGLAVLAVVVIGAVVAAVMCRRKSSGGKGGSYSQAACSDSAQGSDVSLTA

SEQ ID NO: 8 - protein, 366 aa, Homo sapiens
MRVMAPRTLILLLSGALALTETWACSHSMKYFFTSVSRPGRGEPRFISVGYVDDTQFVRFDSDAASPRGEPRAPWVEQEGPEYWDRETQKYKRQAQTDRVSLRNLRGYYNQSEAGSHTLQWMCGCDLGPDGRLLRGYDQYAYDGKDYIALNEDLRSWTAADTAAQITQRKWEAAREAEQRRAYLEGTCVEWLRRYLENGKETLQRAEHPKTHVTHHPVSDHEATLRCWALGFYPAEITLTWQWDGEDQTQDTELVETRPAGDGTFQKWAAVMVPSGEEQRYTCHVQHEGLPEPLTLRWEPSSQPTIPIVGIVAGLAVLAVLAVLGAVVAVVMCRRKSSGGKGGSCSQAASSNSAQGSDESLIACKA

SEQ ID NO: 9 - protein, 358 aa, Homo sapiens [sequence omitted]

SEQ ID NO: 10 - protein, 346 aa, Homo sapiens
MAPRSLLLLLSGALALTDTWAGSHSLRYFSTAVSRPGRGEPRYIAVEYVDDTQFLRFDSDAAIPRMEPREPWVEQEGPQYWEWTTGYAKANAQTDRVALRNLLRRYNQSEAGSHTLQGMNGCDMGPDGRLLRGYHQHAYDGKDYISLNEDLRSWTAADTVAQITQRFYEAEEYAEEFRTYLEGECLELLRRYLENGKETLQRADPPKAHVAHHPISDHEATLRCWALGFYPAEITLTWQRDGEEQTQDTELVETRPAGDGTFQKWAAVVVPSGEEQRYTCHVQHEGLPQPLILRWEQSPQPTIPIVGIVAGLVVLGAVVTGAVVAAVMWRKKSSDRNRGSYSQAAV

SEQ ID NO: 11 - protein, 338 aa, Homo sapiens
MVVMAPRTLFLLLSGALTLTETWAGSHSMRYFSAAVSRPGRGEPRFIAMGYVDDTQFVRFDSDSACPRMEPRAPWVEQEGPEYWEEETRNTKAHAQTDRMNLQTLRGYYNQSEASSHTLQWMIGCDLGSDGRLLRGYEQYAYDGKDYLALNEDLRSWTAADTAAQISKRKCEAANVAEQRRAYLEGTCVEWLHRYLENGKEMLQRADPPKTHVTHHPVFDYEATLRCWALGFYPAEIILTWQRDGEDQTQDVELVETRPAGDGTFQKWAAVVVPSGEEQRYTCHVQHEGLPEPLMLRWKQSSLPTIPIMGIVAGLVVLAAVVTGAAVAAVLWRKKSSD

SEQ ID NO: 12 - protein, 363 aa, Homo sapiens
  MISC_FEATURE (363)..(363): Xaa = any amino acid
MVLMAPRTLLLLLSGALALTQTWARSHSMRYFYTTMSRPGRGEPRFISVGYVDDTQFVRFDSDAASQRMEPRAPWMEREGPEYWDRNTQICKAQAQTERENLRIALRYYNQSEGGSHTMQVMYGCDVGPDGRFLRGYEQHAYDSKDYIALNEDLRSWTAADMAAQITKRKWEAARQAEQLRAYLEGEFVEWLRRYLENGKETLQRADPPKTHMTHHPISDHEATLRCWALGFYPAEITLTWQRDGEDQTHTRSSWRPGLQGMEPSRSGRLWWCLLERSRDTPAMCSMRVCQSPSPDGSHLPSPPSPSWASLLAWFYLLWSLELWSLLCGGRRAQIEKEGATLRLQAATVPRALMCLSRRESVX

SEQ ID NO: 13 - protein, 356 aa, Homo sapiens
MGSWRPEPSSCCSRGPWPWPRPGRAPTPGISAPPFPGRAAGSPASLPWATWTTRSSCGSTVTPVGRRGRGGWSRRGRSIGTYRHWAPRPRHRLTETCGPCSATTTRARRGITSSRECLAATWGPTGVSSAGMSSMPTTARITSPTRTCAPGPPRIPRLRLPSASMRRPMWLSKGEPTWRAPAWSGSADTWRTGRRRCSARTPPKTHVTHPPLTGITRSWVLGFYPAEITLTWQRDGEDQTQDMELVETRPTGDGTFQKWAVVVVPSGEEQRYTCHVQHKGLPKPLILRWEPSPQPTIPIVGIIAGLVLLGAVVTGAVVTAVMWRKKSSDRKGGSYSQAASSQSAQGSDVSLTACKV

SEQ ID NO: 14 - protein, 357 aa, Homo sapiens
MGSWRPEPSSCCSWGPWPPRPGRVPTPGISAPPCPGRVAGSPGTSQWATWTTRSSCGSTATRRLRGCSRSRRGWSRRDRSIGTGAHGTSGPRTDQETCPCRAATTTRARPGLTPSRCMAATWGWKGASSAGMNSTPTMARITPGTRTCAPGPRRTWRLRSPSASGRQKNLQSRSGPTWRARAWRGSQTPGEREGDAAAHGPLPQTHMIHHSVSDYKATLRCWALGFYPVEITLAWQQDGEDQTRDMELLETRPAGDGTFQKWAAVVVPSGEEQRYPCHVQHEGLPKPLTLRWEQSSQPTIPIVGIVAGLVLLGAVVTGAVVSAVMCRKKNSDRVSYSEAASSDHAQGSDVSLTACKV

SEQ ID NO: 15 - protein, 357 aa, Homo sapiens
  MISC_FEATURE (357)..(357): Xaa = any amino acid
MGVMAPRTLLLLLLGALALTETWAGSHSLRYFSTAVSQPGRGEPRFIAVGYVDDTEFVRFDSDSVSPRMERRAPWVEQEGLEYWDQETRNAKGHAQIYRVNLRTLLRYYNQSEAGSHTIQRKHGCDVGPTGASSAGMNSSPTMARITSPTRTCTPGPPRTQRLRSPSTSGKRTNTQSRSGPTGQVHGVAPQTPGEREGDAAARGSPKGTCDPAPHLPGHPEVLGPGPLPCGDHTDLAAGWGGPDPGHGACGDQACRGRNLPEVGGCSGAFRRGAEIHVPCAAGAARAPHPEMGAVFSAHHPHRGHRCWPVSPWSCGHWSCGCCCDVEEEKLRNKEELCSGCLQQLCSVLCISYLSLX

SEQ ID NO: 16 - protein, 9 aa, Artificial Sequence
  Positional scanning library sequence
GLYNTVATL

SEQ ID NO: 17 - protein, 9 aa, Artificial Sequence
  Positional scanning library sequence
PLYNTVATL

SEQ ID NO: 18 - protein, 9 aa, Artificial Sequence
  Positional scanning library sequence
ALYNTVATL

SEQ ID NO: 19 - protein, 9 aa, Artificial Sequence
  Positional scanning library sequence
VLYNTVATL

SEQ ID NO: 20 - protein, 9 aa, Artificial Sequence
  Positional scanning library sequence
LLYNTVATL

SEQ ID NO: 21 - protein, 9 aa, Artificial Sequence
  Positional scanning library sequence
ILYNTVATL

SEQ ID NO: 22 - protein, 9 aa, Artificial Sequence
  Positional scanning library sequence
MLYNTVATL

SEQ ID NO: 23 - protein, 9 aa, Artificial Sequence
  Positional scanning library sequence
FLYNTVATL

SEQ ID NO: 24 - protein, 9 aa, Artificial Sequence
  Positional scanning library sequence
YLYNTVATL

SEQ ID NO: 25 - protein, 9 aa, Artificial Sequence
  Positional scanning library sequence
WLYNTVATL

SEQ ID NO: 26 - protein, 9 aa, Artificial Sequence
  Positional scanning library sequence
HLYNTVATL

SEQ ID NO: 27 - protein, 9 aa, Artificial Sequence
  Positional scanning library sequence
KLYNTVATL

SEQ ID NO: 28 - protein, 9 aa, Artificial Sequence
  Positional scanning library sequence
RLYNTVATL

SEQ ID NO: 29 - protein, 9 aa, Artificial Sequence
  Positional scanning library sequence
QLYNTVATL

SEQ ID NO: 30 - protein, 9 aa, Artificial Sequence
  Positional scanning library sequence
NLYNTVATL

SEQ ID NO: 31 - protein, 9 aa, Artificial Sequence
  Positional scanning library sequence
ELYNTVATL

SEQ ID NO: 32 - protein, 9 aa, Artificial Sequence
  Positional scanning library sequence
DLYNTVATL

SEQ ID NO: 33 - protein, 9 aa, Artificial Sequence
  Positional scanning library sequence
TLYNTVATL

SEQ ID NO: 34 - protein, 9 aa, Artificial Sequence
  Positional scanning library sequence
SGYNTVATL

SEQ ID NO: 35 - protein, 9 aa, Artificial Sequence
  Positional scanning library sequence
SPYNTVATL

SEQ ID NO: 36 - protein, 9 aa, Artificial Sequence
  Positional scanning library sequence
SAYNTVATL

SEQ ID NO: 37 - protein, 9 aa, Artificial Sequence
  Positional scanning library sequence
SVYNTVATL

SEQ ID NO: 38 - protein, 9 aa, Artificial Sequence
  Positional scanning library sequence
SIYNTVATL

SEQ ID NO: 39 - protein, 9 aa, Artificial Sequence
  Positional scanning library sequence
SMYNTVATL

SEQ ID NO: 40 - protein, 9 aa, Artificial Sequence
  Positional scanning library sequence
SFYNTVATL

SEQ ID NO: 41 - protein, 9 aa, Artificial Sequence
  Positional scanning library sequence
SYYNTVATL

SEQ ID NO: 42 - protein, 9 aa, Artificial Sequence
  Positional scanning library sequence
SWYNTVATL

SEQ ID NO: 43 - protein, 9 aa, Artificial Sequence
  Positional scanning library sequence
SHYNTVATL

SEQ ID NO: 44 - protein, 9 aa, Artificial Sequence
  Positional scanning library sequence
SKYNTVATL

SEQ ID NO: 45 - protein, 9 aa, Artificial Sequence
  Positional scanning library sequence
SRYNTVATL

SEQ ID NO: 46 - protein, 9 aa, Artificial Sequence
  Positional scanning library sequence
SQYNTVATL

SEQ ID NO: 47 - protein, 9 aa, Artificial Sequence
  Positional scanning library sequence
SNYNTVATL

SEQ ID NO: 48 - protein, 9 aa, Artificial Sequence
  Positional scanning library sequence
SEYNTVATL

SEQ ID NO: 49 - protein, 9 aa, Artificial Sequence
  Positional scanning library sequence
SDYNTVATL

SEQ ID NO: 50 - protein, 9 aa, Artificial Sequence
  Positional scanning library sequence
SSYNTVATL

SEQ ID NO: 51 - protein, 9 aa, Artificial Sequence
  Positional scanning library sequence
STYNTVATL

SEQ ID NO: 52 - protein, 9 aa, Artificial Sequence
  Positional scanning library sequence
SLGNTVATL

SEQ ID NO: 53 - protein, 9 aa, Artificial Sequence
  Positional scanning library sequence
SLPNTVATL

SEQ ID NO: 54 - protein, 9 aa, Artificial Sequence
  Positional scanning library sequence
SLANTVATL

SEQ ID NO: 55 - protein, 9 aa, Artificial Sequence
  Positional scanning library sequence
SLVNTVATL

SEQ ID NO: 56 - protein, 9 aa, Artificial Sequence
  Positional scanning library sequence
SLLNTVATL

SEQ ID NO: 57 - protein, 9 aa, Artificial Sequence
  Positional scanning library sequence
SLINTVATL

SEQ ID NO: 58 - protein, 9 aa, Artificial Sequence
  Positional scanning library sequence
SLMNTVATL

SEQ ID NO: 59 - protein, 9 aa, Artificial Sequence
  Positional scanning library sequence
SLFNTVATL

SEQ ID NO: 60 - protein, 9 aa, Artificial Sequence
  Positional scanning library sequence
SLWNTVATL

SEQ ID NO: 61 - protein, 9 aa, Artificial Sequence
  Positional scanning library sequence
SLHNTVATL

SEQ ID NO: 62 - protein, 9 aa, Artificial Sequence
  Positional scanning library sequence
SLKNTVATL

SEQ ID NO: 63 - protein, 9 aa, Artificial Sequence
  Positional scanning library sequence
SLRNTVATL

SEQ ID NO: 64 - protein, 9 aa, Artificial Sequence
  Positional scanning library sequence
SLQNTVATL

SEQ ID NO: 65 - protein, 9 aa, Artificial Sequence
  Positional scanning library sequence
SLNNTVATL

SEQ ID NO: 66 - protein, 9 aa, Artificial Sequence
  Positional scanning library sequence
SLENTVATL

SEQ ID NO: 67 - protein, 9 aa, Artificial Sequence
  Positional scanning library sequence
SLDNTVATL

SEQ ID NO: 68 - protein, 9 aa, Artificial Sequence
  Positional scanning library sequence
SLSNTVATL

SEQ ID NO: 69 - protein, 9 aa, Artificial Sequence
  Positional scanning library sequence
SLTNTVATL

SEQ ID NO: 70 - protein, 9 aa, Artificial Sequence
  Positional scanning library sequence
SLYGTVATL

SEQ ID NO: 71 - protein, 9 aa, Artificial Sequence
  Positional scanning library sequence
SLYPTVATL

SEQ ID NO: 72 - protein, 9 aa, Artificial Sequence
  Positional scanning library sequence
SLYATVATL

SEQ ID NO: 73 - protein, 9 aa, Artificial Sequence
  Positional scanning library sequence
SLYVTVATL

SEQ ID NO: 74 - protein, 9 aa, Artificial Sequence
  Positional scanning library sequence
SLYLTVATL

SEQ ID NO: 75 - protein, 9 aa, Artificial Sequence
  Positional scanning library sequence
SLYITVATL

SEQ ID NO: 76 - protein, 9 aa, Artificial Sequence
  Positional scanning library sequence
SLYMTVATL

SEQ ID NO: 77 - protein, 9 aa, Artificial Sequence
  Positional scanning library sequence
SLYFTVATL

SEQ ID NO: 78 - protein, 9 aa, Artificial Sequence
  Positional scanning library sequence
SLYYTVATL

SEQ ID NO: 79 - protein, 9 aa, Artificial Sequence
  Positional scanning library sequence
SLYWTVATL

SEQ ID NO: 80 - protein, 9 aa, Artificial Sequence
  Positional scanning library sequence
SLYHTVATL

SEQ ID NO: 81 - protein, 9 aa, Artificial Sequence
  Positional scanning library sequence
SLYKTVATL

SEQ ID NO: 82 - protein, 9 aa, Artificial Sequence
  Positional scanning library sequence
SLYRTVATL

SEQ ID NO: 83 - protein, 9 aa, Artificial Sequence
  Positional scanning library sequence
SLYQTVATL

SEQ ID NO: 84 - protein, 9 aa, Artificial Sequence
  Positional scanning library sequence
SLYETVATL

SEQ ID NO: 85 - protein, 9 aa, Artificial Sequence
  Positional scanning library sequence
SLYDTVATL

SEQ ID NO: 86 - protein, 9 aa, Artificial Sequence
  Positional scanning library sequence
SLYSTVATL

SEQ ID NO: 87 - protein, 9 aa, Artificial Sequence
  Positional scanning library sequence
SLYTTVATL

SEQ ID NO: 88 - protein, 9 aa, Artificial Sequence
  Positional scanning library sequence
SLYNGVATL

SEQ ID NO: 89 - protein, 9 aa, Artificial Sequence
  Positional scanning library sequence
SLYNPVATL

SEQ ID NO: 90 - protein, 9 aa, Artificial Sequence
  Positional scanning library sequence
SLYNAVATL

SEQ ID NO: 91 - protein, 9 aa, Artificial Sequence
  Positional scanning library sequence
SLYNVVATL

SEQ ID NO: 92 - protein, 9 aa, Artificial Sequence
  Positional scanning library sequence
SLYNLVATL

SEQ ID NO: 93 - protein, 9 aa, Artificial Sequence
  Positional scanning library sequence
SLYNIVATL

SEQ ID NO: 94 - protein, 9 aa, Artificial Sequence
  Positional scanning library sequence
SLYNMVATL

SEQ ID NO: 95 - protein, 9 aa, Artificial Sequence
  Positional scanning library sequence
SLYNFVATL

SEQ ID NO: 96 - protein, 9 aa, Artificial Sequence
  Positional scanning library sequence
SLYNYVATL

SEQ ID NO: 97 - protein, 9 aa, Artificial Sequence
  Positional scanning library sequence
SLYNWVATL

SEQ ID NO: 98 - protein, 9 aa, Artificial Sequence
  Positional scanning library sequence
SLYNHVATL

SEQ ID NO: 99 - protein, 9 aa, Artificial Sequence
  Positional scanning library sequence
SLYNKVATL

SEQ ID NO: 100 - protein, 9 aa, Artificial Sequence
  Positional scanning library sequence
SLYNRVATL

SEQ ID NO: 101 - protein, 9 aa, Artificial Sequence
  Positional scanning library sequence
SLYNQVATL

SEQ ID NO: 102 - protein, 9 aa, Artificial Sequence
  Positional scanning library sequence
SLYNNVATL

SEQ ID NO: 103 - protein, 9 aa, Artificial Sequence
  Positional scanning library sequence
SLYNEVATL

SEQ ID NO: 104 - protein, 9 aa, Artificial Sequence
  Positional scanning library sequence
SLYNDVATL

SEQ ID NO: 105 - protein, 9 aa, Artificial Sequence
  Positional scanning library sequence
SLYNSVATL

SEQ ID NO: 106 - protein, 9 aa, Artificial Sequence
  Positional scanning library sequence
SLYNTGATL

SEQ ID NO: 107 - protein, 9 aa, Artificial Sequence
  Positional scanning library sequence
SLYNTPATL

SEQ ID NO: 108 - protein, 9 aa, Artificial Sequence
  Positional scanning library sequence
SLYNTAATL

SEQ ID NO: 109 - protein, 9 aa, Artificial Sequence
  Positional scanning library sequence
SLYNTLATL

SEQ ID NO: 110 - protein, 9 aa, Artificial Sequence
  Positional scanning library sequence
SLYNTIATL

SEQ ID NO: 111 - protein, 9 aa, Artificial Sequence
  Positional scanning library sequence
SLYNTMATL

SEQ ID NO: 112 - protein, 9 aa, Artificial Sequence
  Positional scanning library sequence
SLYNTFATL

SEQ ID NO: 113 - protein, 9 aa, Artificial Sequence
  Positional scanning library sequence
SLYNTYATL

SEQ ID NO: 114 - protein, 9 aa, Artificial Sequence
  Positional scanning library sequence
SLYNTWATL

SEQ ID NO: 115 - protein, 9 aa, Artificial Sequence
  Positional scanning library sequence
SLYNTHATL

SEQ ID NO: 116 - protein, 9 aa, Artificial Sequence
  Positional scanning library sequence
SLYNTKATL

SEQ ID NO: 117 - protein, 9 aa, Artificial Sequence
  Positional scanning library sequence
SLYNTRATL

SEQ ID NO: 118 - protein, 9 aa, Artificial Sequence
  Positional scanning library sequence
SLYNTQATL

SEQ ID NO: 119 - protein, 9 aa, Artificial Sequence
  Positional scanning library sequence
SLYNTNATL

SEQ ID NO: 120 - protein, 9 aa, Artificial Sequence
  Positional scanning library sequence
SLYNTEATL

SEQ ID NO: 121 - protein, 9 aa, Artificial Sequence
  Positional scanning library sequence
SLYNTDATL

SEQ ID NO: 122 - protein, 9 aa, Artificial Sequence
  Positional scanning library sequence
SLYNTSATL

SEQ ID NO: 123 - protein, 9 aa, Artificial Sequence
  Positional scanning library sequence
SLYNTTATL

SEQ ID NO: 124 - protein, 9 aa, Artificial Sequence
  Positional scanning library sequence
SLYNTVGTL

SEQ ID NO: 125 - protein, 9 aa, Artificial Sequence
  Positional scanning library sequence
SLYNTVPTL

SEQ ID NO: 126 - protein, 9 aa, Artificial Sequence
  Positional scanning library sequence
SLYNTVVTL

SEQ ID NO: 127 - protein, 9 aa, Artificial Sequence
  Positional scanning library sequence
SLYNTVLTL

SEQ ID NO: 128 - protein, 9 aa, Artificial Sequence
  Positional scanning library sequence
SLYNTVITL

SEQ ID NO: 129 - protein, 9 aa, Artificial Sequence
  Positional scanning library sequence
SLYNTVMTL

SEQ ID NO: 130 - protein, 9 aa, Artificial Sequence
  Positional scanning library sequence
SLYNTVFTL

SEQ ID NO: 131 - protein, 9 aa, Artificial Sequence
  Positional scanning library sequence
SLYNTVYTL

SEQ ID NO: 132 - protein, 9 aa, Artificial Sequence
  Positional scanning library sequence
SLYNTVWTL

SEQ ID NO: 133 - protein, 9 aa, Artificial Sequence
  Positional scanning library sequence
SLYNTVHTL

SEQ ID NO: 134 - protein, 9 aa, Artificial Sequence
  Positional scanning library sequence
SLYNTVKTL

SEQ ID NO: 135 - protein, 9 aa, Artificial Sequence
  Positional scanning library sequence
SLYNTVRTL

SEQ ID NO: 136 - protein, 9 aa, Artificial Sequence
  Positional scanning library sequence
SLYNTVQTL

SEQ ID NO: 137 - protein, 9 aa, Artificial Sequence
  Positional scanning library sequence
SLYNTVNTL

SEQ ID NO: 138 - protein, 9 aa, Artificial Sequence
  Positional scanning library sequence
SLYNTVETL

SEQ ID NO: 139 - protein, 9 aa, Artificial Sequence
  Positional scanning library sequence
SLYNTVDTL

SEQ ID NO: 140 - protein, 9 aa, Artificial Sequence
  Positional scanning library sequence
SLYNTVSTL

SEQ ID NO: 141 - protein, 9 aa, Artificial Sequence
  Positional scanning library sequence
SLYNTVTTL

SEQ ID NO: 142 - protein, 9 aa, Artificial Sequence
  Positional scanning library sequence
SLYNTVAGL

SEQ ID NO: 143 - protein, 9 aa, Artificial Sequence
  Positional scanning library sequence
SLYNTVAPL

SEQ ID NO: 144 - protein, 9 aa, Artificial Sequence
  Positional scanning library sequence
SLYNTVAAL

SEQ ID NO: 145 - protein, 9 aa, Artificial Sequence
  Positional scanning library sequence
SLYNTVAVL

SEQ ID NO: 146 - protein, 9 aa, Artificial Sequence
  Positional scanning library sequence
SLYNTVALL

SEQ ID NO: 147 - protein, 9 aa, Artificial Sequence
  Positional scanning library sequence
SLYNTVAIL

SEQ ID NO: 148 - protein, 9 aa, Artificial Sequence
  Positional scanning library sequence
SLYNTVAML

SEQ ID NO: 149 - protein, 9 aa, Artificial Sequence
  Positional scanning library sequence
SLYNTVAFL

SEQ ID NO: 150 - protein, 9 aa, Artificial Sequence
  Positional scanning library sequence
SLYNTVAYL

SEQ ID NO: 151 - protein, 9 aa, Artificial Sequence
  Positional scanning library sequence
SLYNTVAWL

SEQ ID NO: 152 - protein, 9 aa, Artificial Sequence
  Positional scanning library sequence
SLYNTVAHL

SEQ ID NO: 153 - protein, 9 aa, Artificial Sequence
  Positional scanning library sequence
SLYNTVAKL

SEQ ID NO: 154 - protein, 9 aa, Artificial Sequence
  Positional scanning library sequence
SLYNTVARL

SEQ ID NO: 155 - protein, 9 aa, Artificial Sequence
  Positional scanning library sequence
SLYNTVAQL

SEQ ID NO: 156 - protein, 9 aa, Artificial Sequence
  Positional scanning library sequence
SLYNTVANL

SEQ ID NO: 157 - protein, 9 aa, Artificial Sequence
  Positional scanning library sequence
SLYNTVAEL

SEQ ID NO: 158 - protein, 9 aa, Artificial Sequence
  Positional scanning library sequence
SLYNTVADL

SEQ ID NO: 159 - protein, 9 aa, Artificial Sequence
  Positional scanning library sequence
SLYNTVASL

SEQ ID NO: 160 - protein, 9 aa, Artificial Sequence
  Positional scanning library sequence
SLYNTVATG

SEQ ID NO: 161 - protein, 9 aa, Artificial Sequence
  Positional scanning library sequence
SLYNTVATP

SEQ ID NO: 162 - protein, 9 aa, Artificial Sequence
  Positional scanning library sequence
SLYNTVATA

SEQ ID NO: 163 - protein, 9 aa, Artificial Sequence
  Positional scanning library sequence
SLYNTVATV

SEQ ID NO: 164 - protein, 9 aa, Artificial Sequence
  Positional scanning library sequence
SLYNTVATI

SEQ ID NO: 165 - protein, 9 aa, Artificial Sequence
  Positional scanning library sequence
SLYNTVATM

SEQ ID NO: 166 - protein, 9 aa, Artificial Sequence
  Positional scanning library sequence
SLYNTVATF

SEQ ID NO: 167 - protein, 9 aa, Artificial Sequence
  Positional scanning library sequence
SLYNTVATY

SEQ ID NO: 168 - protein, 9 aa, Artificial Sequence
  Positional scanning library sequence
SLYNTVATW

SEQ ID NO: 169 - protein, 9 aa, Artificial Sequence
  Positional scanning library sequence
SLYNTVATH

SEQ ID NO: 170 - protein, 9 aa, Artificial Sequence
  Positional scanning library sequence
SLYNTVATK

SEQ ID NO: 171 - protein, 9 aa, Artificial Sequence
  Positional scanning library sequence
SLYNTVATR

SEQ ID NO: 172 - protein, 9 aa, Artificial Sequence
  Positional scanning library sequence
SLYNTVATQ

SEQ ID NO: 173 - protein, 9 aa, Artificial Sequence
  Positional scanning library sequence
SLYNTVATN

SEQ ID NO: 174 - protein, 9 aa, Artificial Sequence
  Positional scanning library sequence
SLYNTVATE

SEQ ID NO: 175 - protein, 9 aa, Artificial Sequence
  Positional scanning library sequence
SLYNTVATD

SEQ ID NO: 176 - protein, 9 aa, Artificial Sequence
  Positional scanning library sequence
SLYNTVATS

SEQ ID NO: 177 - protein, 9 aa, Artificial Sequence
  Positional scanning library sequence
SLYNTVATT

SEQ ID NO: 178 - protein, 9 aa, Homo sapiens
RVYNTVPLV

SEQ ID NO: 179 - protein, 9 aa, Homo sapiens
RMYNLVSRI

SEQ ID NO: 180 - protein, 9 aa, Homo sapiens
SLYNMVPSI

SEQ ID NO: 181 - protein, 9 aa, Homo sapiens
TVYNMVPSI

SEQ ID NO: 182 - protein, 9 aa, Homo sapiens
ALYNVIAMA

SEQ ID NO: 183 - protein, 9 aa, Homo sapiens
AIYNLLPDI

SEQ ID NO: 184 - protein, 9 aa, Homo sapiens
STYNLVSTS

SEQ ID NO: 185 - protein, 9 aa, Homo sapiens
SVYNMVPSI

SEQ ID NO: 186 - protein, 9 aa, Homo sapiens
RTYNVLAIL

SEQ ID NO: 187 - protein, 9 aa, Homo sapiens
SVYNLVSIA

SEQ ID NO: 188 - protein, 9 aa, Homo sapiens
RAYNLIGTV

SEQ ID NO: 189 - protein, 9 aa, Homo sapiens
ALFNLIPVG

SEQ ID NO: 190 - protein, 9 aa, Homo sapiens
RIYNVIGTL

SEQ ID NO: 191 - protein, 9 aa, Homo sapiens
RIYNVVGTI

SEQ ID NO: 192 - protein, 9 aa, Homo sapiens
TLFNLVPNS

SEQ ID NO: 193 - protein, 9 aa, Homo sapiens
SLFNVISIL

SEQ ID NO: 194 - protein, 9 aa, Homo sapiens
STFNLVAIS

SEQ ID NO: 195 - protein, 9 aa, Homo sapiens
TLFNLIPVG

SEQ ID NO: 196 - protein, 9 aa, Homo sapiens
TIFNLIPNS

SEQ ID NO: 197 - protein, 9 aa, Homo sapiens
ALYNVLAKV

SEQ ID NO: 198 - protein, 9 aa, Homo sapiens
AVFNLLPHT

SEQ ID NO: 199 - protein, 9 aa, Homo sapiens
RMYNLLGHM

SEQ ID NO: 200 - protein, 9 aa, Homo sapiens
STWNTPPNM

SEQ ID NO: 201 - protein, 9 aa, Homo sapiens
NIYNLIAII

SEQ ID NO: 202 - protein, 9 aa, Homo sapiens
RIYNLPPEL

SEQ ID NO: 203 - protein, 9 aa, Homo sapiens
TTFNLPSAA

SEQ ID NO: 204 - protein, 9 aa, Homo sapiens
MFFNVIAIV

SEQ ID NO: 205 - protein, 9 aa, Homo sapiens
SLWNTVSGI

SEQ ID NO: 206 - protein, 9 aa, Homo sapiens
MLWNLLALR

SEQ ID NO: 207 - protein, 9 aa, Homo sapiens
VFWNLLPTV

SEQ ID NO: 208 - protein, 9 aa, Homo sapiens
STFNTTSNG

SEQ ID NO: 209 - protein, 9 aa, Homo sapiens
GFFNLLSHV

SEQ ID NO: 210 - protein, 9 aa, Homo sapiens
LLYNVPAVA

SEQ ID NO: 211 - protein, 9 aa, Homo sapiens
ALFNTISQG

SEQ ID NO: 212 - protein, 9 aa, Homo sapiens
TTFNTLAGS

SEQ ID NO: 213 - protein, 9 aa, Homo sapiens
SLWNLLGNA

SEQ ID NO: 214 - protein, 9 aa, Homo sapiens
SLYNLLNLT

SEQ ID NO: 215 - protein, 9 aa, Homo sapiens
GVWNLLSIV

SEQ ID NO: 216 - protein, 9 aa, Homo sapiens
ALFNVVNSI

SEQ ID NO: 217 - protein, 9 aa, Homo sapiens
VIYNLLGLA

SEQ ID NO: 218 - protein, 9 aa, Homo sapiens
SIFNIVAIA

SEQ ID NO: 219 - protein, 9 aa, Homo sapiens
TVYNTVSEG

SEQ ID NO: 220 - protein, 9 aa, Homo sapiens
DLWNTLSSL

SEQ ID NO: 221 - protein, 9 aa, Homo sapiens
IFFNLLAVL

SEQ ID NO: 222 - protein, 9 aa, Homo sapiens
DLFNLLPDV

SEQ ID NO: 223 - protein, 9 aa, Homo sapiens
LSWNVVPNA

SEQ ID NO: 224 - protein, 9 aa, Homo sapiens
MLWNLLALH

SEQ ID NO: 225 - protein, 9 aa, Homo sapiens
TIFNTVNTS

SEQ ID NO: 226 - protein, 9 aa, Homo sapiens
KTFNLIPAV

SEQ ID NO: 227 - protein, 9 aa, Homo sapiens
NLFNVTPLI

SEQ ID NO: 228 - protein, 9 aa, Homo sapiens
SYWNIISTV

SEQ ID NO: 229 - protein, 9 aa, Homo sapiens
GVFNLIAVL

SEQ ID NO: 230 - protein, 9 aa, Homo sapiens
RLFNITSSA

SEQ ID NO: 231 - protein, 9 aa, Homo sapiens
NLWNLVAVI

SEQ ID NO: 232 - protein, 9 aa, Homo sapiens
RIFNLIGMM

SEQ ID NO: 233 - protein, 9 aa, Homo sapiens
RLFNVVSRG

SEQ ID NO: 234 - protein, 9 aa, Homo sapiens
LVFNVIPTL

SEQ ID NO: 235 - protein, 9 aa, Homo sapiens
TTWNILSSA

SEQ ID NO: 236 - protein, 9 aa, Homo sapiens
KLFNVLSTL

SEQ ID NO: 237 - protein, 9 aa, Homo sapiens
RVYNLTAKS

SEQ ID NO: 238 - protein, 9 aa, Homo sapiens
LTFNTISLS

SEQ ID NO: 239 - protein, 9 aa, Homo sapiens
AQFNLLSST

SEQ ID NO: 240 - protein, 9 aa, Homo sapiens
VVYNVLSEL

SEQ ID NO: 241 - protein, 9 aa, Homo sapiens
KVYNTPSTS

SEQ ID NO: 242 - protein, 9 aa, Homo sapiens
GIFNIIPST

SEQ ID NO: 243 - protein, 9 aa, Homo sapiens
NIYNTLSGL

SEQ ID NO: 244 - protein, 9 aa, Homo sapiens
RLFNLTSTF

SEQ ID NO: 245 - protein, 9 aa, Homo sapiens
TVWNTLSSL

SEQ ID NO: 246 - protein, 9 aa, Homo sapiens
RLFNMLSAV

SEQ ID NO: 247 - protein, 9 aa, Homo sapiens
SIWNVTAIA

SEQ ID NO: 248 - protein, 9 aa, Homo sapiens
ALFNLMSGI

SEQ ID NO: 249 - protein, 9 aa, Homo sapiens
IVYNLLSAM

SEQ ID NO: 250 - protein, 9 aa, Homo sapiens
ISFNMLPSI

SEQ ID NO: 251 - protein, 9 aa, Homo sapiens
NTYNILPGS

SEQ ID NO: 252 - protein, 9 aa, Homo sapiens
RLWNMVNVT

SEQ ID NO: 253 - protein, 9 aa, Homo sapiens
SAFNITSLI

SEQ ID NO: 254 - protein, 9 aa, Homo sapiens
NIFNLPNIV

SEQ ID NO: 255 - protein, 9 aa, Homo sapiens
GVYNLPGAS

SEQ ID NO: 256 - protein, 9 aa, Homo sapiens
GTYNVISLV

SEQ ID NO: 257 - protein, 9 aa, Homo sapiens
SIFNTLSDI

SEQ ID NO: 258 - protein, 9 aa, Homo sapiens
TIFNILSGI

SEQ ID NO: 259 - protein, 9 aa, Homo sapiens
LLFNLISSS

SEQ ID NO: 260 - protein, 9 aa, Homo sapiens
RTFNLTAGS

SEQ ID NO: 261 - protein, 9 aa, Homo sapiens
TVFNILPGG

SEQ ID NO: 262 - protein, 9 aa, Homo sapiens
GLFNIPPAS

SEQ ID NO: 263 - protein, 9 aa, Homo sapiens
RMFNIISDS

SEQ ID NO: 264 - protein, 9 aa, Homo sapiens
TTFNIVGTT

SEQ ID NO: 265 - protein, 9 aa, Homo sapiens
ALFNLMSGV

SEQ ID NO: 266 - protein, 9 aa, Homo sapiens
SVFNITAIA

SEQ ID NO: 267 - protein, 9 aa, Homo sapiens
KIYNTPSAS

SEQ ID NO: 268 - protein, 9 aa, Homo sapiens
LLYNLLGSS

SEQ ID NO: 269 - protein, 9 aa, Homo sapiens
SLYNMMGEA

SEQ ID NO: 270 - protein, 9 aa, Homo sapiens
SLWNLMGNA

SEQ ID NO: 271 - protein, 9 aa, Homo sapiens
GLYNIVGNA

SEQ ID NO: 272 - protein, 9 aa, Homo sapiens
LTWNLTPKA

SEQ ID NO: 273 - protein, 9 aa, Homo sapiens
LIFNVTGLA

SEQ ID NO: 274 - protein, 9 aa, Homo sapiens
SIFNITGIA

SEQ ID NO: 275 - protein, 9 aa, Homo sapiens
LTFNLVSDA

SEQ ID NO: 276 - protein, 9 aa, Homo sapiens
MQWNILAQA

SEQ ID NO: 277 - protein, 9 aa, Homo sapiens
LSWNLVPEA

SEQ ID NO: 278 - protein, 9 aa, Homo sapiens
DLWNTLSEA

SEQ ID NO: 279 - protein, 9 aa, Homo sapiens
GLFNIPPAF

SEQ ID NO: 280 - protein, 9 aa, Homo sapiens
LIWNILASF

SEQ ID NO: 281 - protein, 9 aa, Homo sapiens
LLFNMLPGG

SEQ ID NO: 282 - protein, 9 aa, Homo sapiens
LVYNIMSSG

SEQ ID NO: 283 - protein, 9 aa, Homo sapiens
IIYNVPGTG

SEQ ID NO: 284 - protein, 9 aa, Homo sapiens
VIYNVTSDG

SEQ ID NO: 285 - protein, 9 aa, Homo sapiens
GTFNLPSDG

SEQ ID NO: 286 - protein, 9 aa, Homo sapiens
KLWNTLNLI

SEQ ID NO: 287 - protein, 9 aa, Homo sapiens
LMWNIISII

SEQ ID NO: 288 - protein, 9 aa, Homo sapiens
GLFNTTSNI

SEQ ID NO: 289 - protein, 9 aa, Homo sapiens
LIFNTLSLI

SEQ ID NO: 290 - protein, 9 aa, Homo sapiens
SVFNLMNAI

SEQ ID NO: 291 - protein, 9 aa, Homo sapiens
LTFNILGQI

SEQ ID NO: 292 - protein, 9 aa, Homo sapiens
GLFNMVSSL

SEQ ID NO: 293 - protein, 9 aa, Homo sapiens
KIFNIINSL

SEQ ID NO: 294 - protein, 9 aa, Homo sapiens
AVWNVLGNL

SEQ ID NO: 295 - protein, 9 aa, Homo sapiens
KVFNIVSDL

SEQ ID NO: 296 - protein, 9 aa, Homo sapiens
DLWNVVSHL

SEQ ID NO: 297 - protein, 9 aa, Homo sapiens
LQFNTVSKL

SEQ ID NO: 298 - protein, 9 aa, Homo sapiens
MSFNTVSEL

SEQ ID NO: 299 - protein, 9 aa, Homo sapiens
ASWNIVNLL

SEQ ID NO: 300 - protein, 9 aa, Homo sapiens
ISFNIISAL

SEQ ID NO: 301 - protein, 9 aa, Homo sapiens
AFFNILNEL

SEQ ID NO: 302 - protein, 9 aa, Homo sapiens
LVFNLLPIM

SEQ ID NO: 303 - protein, 9 aa, Homo sapiens
KIFNTVPDM

SEQ ID NO: 304 - protein, 9 aa, Homo sapiens
MLFNLIGLS

SEQ ID NO: 305 - protein, 9 aa, Homo sapiens
LLFNLPPGS

SEQ ID NO: 306 - protein, 9 aa, Homo sapiens
MTFNLIGES

SEQ ID NO: 307 - protein, 9 aa, Homo sapiens
KVYNIPGIS

SEQ ID NO: 308 - protein, 9 aa, Homo sapiens
GIYNIPGDS

SEQ ID NO: 309 - protein, 9 aa, Homo sapiens
GLYNLMNIT

SEQ ID NO: 310 - protein, 9 aa, Homo sapiens
LTWNMINTT

SEQ ID NO: 311 - protein, 9 aa, Homo sapiens
IVFNVLSDT

SEQ ID NO: 312 - protein, 9 aa, Homo sapiens
IVFNVVSDT

SEQ ID NO: 313 - protein, 9 aa, Homo sapiens
LIFNITASV

SEQ ID NO: 314 - protein, 9 aa, Homo sapiens
IVFNLTNNV

SEQ ID NO: 315 - protein, 9 aa, Homo sapiens
KSFNVLSSV

SEQ ID NO: 316 - protein, 9 aa, Homo sapiens
LAFNILGMV

SEQ ID NO: 317 - protein, 9 aa, Homo sapiens
VSWNITGTV

SEQ ID NO: 318 - protein, 9 aa, Artificial Sequence
  Peptide ligand sequence
SLFNTIAVL

SEQ ID NO: 319 - protein, 8 aa, Artificial Sequence
  Peptide ligand sequence
SLFNTVAV

SEQ ID NO: 320 - protein, 9 aa, Artificial Sequence
  Peptide ligand sequence
SLFNTIATL

SEQ ID NO: 321 - protein, 9 aa, Artificial Sequence
  Peptide ligand sequence
SLYNTIAVL

SEQ ID NO: 322 - protein, 275 aa, Homo sapiens [sequence omitted]

SEQ ID NO: 323 - protein, 275 aa, Artificial sequence
  Y84C/A139C HLA-A*02:01 variant sequence
GSHSMRYFFTSVSRPGRGEPRFIAVGYVDDTQFVRFDSDAASQRMEPRAPWIEQEGPEYWDGETRKVKAHSQTHRVDLGTLRGCYNQSEAGSHTVQRMYGCDVGSDWRFLRGYHQYAYDGKDYIALKEDLRSWTAADMCAQTTKHKWEAAHVAEQLRAYLEGTCVEWLRRYLENGKETLQRTDAPKTHMTHHAVSDHEATLRCWALSFYPAEITLTWQRDGEDQTQDTELVETRPAGDGTFQKWAAVVVPSGQEQRYTCHVQHEGLPKPLTLRWE

SEQ ID NO: 324 - protein, 275 aa, Artificial Sequence
  F22C/S71C HLA-A*02:01 variant
GSHSMRYFFTSVSRPGRGEPRCIAVGYVDDTQFVRFDSDAASQRMEPRAPWIEQEGPEYWDGETRKVKAHCQTHRVDLGTLRGYYNQSEAGSHTVQRMYGCDVGSDWRFLRGYHQYAYDGKDYIALKEDLRSWTAADMAAQTTKHKWEAAHVAEQLRAYLEGTCVEWLRRYLENGKETLQRTDAPKTHMTHHAVSDHEATLRCWALSFYPAEITLTWQRDGEDQTQDTELVETRPAGDGTFQKWAAVVVPSGQEQRYTCHVQHEGLPKPLTLRWE

SEQ ID NO: 325 - protein, 275 aa, Artificial Sequence
  F22C/S71C W51C/G175C HLA-A*02:01 variant
GSHSMRYFFTSVSRPGRGEPRCIAVGYVDDTQFVRFDSDAASQRMEPRAPCIEQEGPEYWDGETRKVKAHCQTHRVDLGTLRGYYNQSEAGSHTVQRMYGCDVGSDWRFLRGYHQYAYDGKDYIALKEDLRSWTAADMAAQTTKHKWEAAHVAEQLRAYLEGTCVEWLRRYLENCKETLQRTDAPKTHMTHHAVSDHEATLRCWALSFYPAEITLTWQRDGEDQTQDTELVETRPAGDGTFQKWAAVVVPSGQEQRYTCHVQHEGLPKPLTLRWE